European Patent Application EP 4 644 410 A1, published November 5, 2025. Title: Recombinant fusion protein having modified cysteine residue for antigen delivery and uses thereof. Applicant: LG CHEM, LTD. The sequence listing filed with the application follows.

SEQUENCE LISTING (90 sequences)

SEQ ID NO: 1 - protein, 27 aa, synthetic construct
  REGION 1..27: note = epitope M30
PSKPSFQEFVDWENVSPELNSTDQPFL

SEQ ID NO: 2 - protein, 27 aa, synthetic construct
  REGION 1..27: note = epitope M44
EFKHIKAFDRTFANNPGPMVVFATPGM

SEQ ID NO: 3 - protein, 27 aa, synthetic construct
  REGION 1..27: note = epitope M12
TPPPEEAMPFEFNGPAQGDHSQPPLQV

SEQ ID NO: 4 - protein, 27 aa, synthetic construct
  REGION 1..27: note = epitope M21
SSPDEVALVEGVQSLGFTYLRLKDNYM

SEQ ID NO: 5 - protein, 17 aa, synthetic construct
  REGION 1..17: note = epitope C5
IYLESVAIMPQLFMVSK

SEQ ID NO: 6 - protein, 27 aa, synthetic construct
  REGION 1..27: note = epitope MelanA
YPKKGHGHSYTTAEELAGIGILTVILG

SEQ ID NO: 7 - protein, 105 aa, synthetic construct
  REGION 1..105: note = hTrx.v1 (human Thioredoxin variant1)
MVKQIESKTAFQEALDAAGDKLVVVDFSATWCGPCKMIKPFFHSLSEKYSNVIFLEVDVDDSQDVASESEVKSMPTFQFFKKGQKVGEFSGANKEKLEATINELV

SEQ ID NO: 8 - protein, 105 aa, synthetic construct
  REGION 1..105: note = hTrx.v2 (human Thioredoxin variant2)
MVKQIESKTAFQEALDAAGDKLVVVDFSATWCGPCKMIKPFFHSLSEKYSNVIFLEVDVDDCQDVASECEVKSMPTFQFFKKGQKVGEFSGANKEKLEATINELV

SEQ ID NO: 9 - protein, 105 aa, synthetic construct
  REGION 1..105: note = hTrx.v3 (human Thioredoxin variant3)
MVKQIESKTAFQEALDAAGDKLVVVDFSATWSGPSKMIKPFFHSLSEKYSNVIFLEVDVDDSQDVASESEVKSMPTFQFFKKGQKVGEFSGANKEKLEATINELV

SEQ ID NO: 10 - protein, 105 aa, synthetic construct
  REGION 1..105: note = hTrx.wt (human Thioredoxin wildtype)
MVKQIESKTAFQEALDAAGDKLVVVDFSATWCGPCKMIKPFFHSLSEKYSNVIFLEVDVDDCQDVASECEVKCMPTFQFFKKGQKVGEFSGANKEKLEATINELV

SEQ ID NO: 11 - protein, 109 aa, synthetic construct
  REGION 1..109: note = TrxA (Escherichia coli, Thioredoxin 1)
MSDKIIHLTDDSFDTDVLKADGAILVDFWAEWCGPCKMIAPILDEIADEYQGKLTVAKLNIDQNPGTAPKYGIRGIPTLLLFKNGEVAATKVGALSKGQLKEFLDANLA

SEQ ID NO: 12 - protein, 109 aa, synthetic construct
  REGION 1..109: note = TrxA.v2(Escherichia coli, Thioredoxin 1 variant 2)
MSDKIIHLTDDSFDTDVLKADGAILVDFWAEWSGPSKMIAPILDEIADEYQGKLTVAKLNIDQNPGTAPKYGIRGIPTLLLFKNGEVAATKVGALSKGQLKEFLDANLA

SEQ ID NO: 13 - protein, 40 aa, synthetic construct
  REGION 1..40: note = PSBD (peripheral subunit-binding domain)?
VIAMPSVRKYAREKGVDIRLVQGTGKNGRVLKEDIDAWLA

SEQ ID NO: 14 - protein, 141 aa, synthetic construct
  REGION 1..141: note = TrxA-M30
MSDKIIHLTDDSFDTDVLKADGAILVDFWAEWCGPCKMIAPILDEIADEYQGKLTVAKLNIDQNPGTAPKYGIRGIPTLLLFKNGEVAATKVGALSKGQLKEFLDANLAGGGGSPSKPSFQEFVDWENVSPELNSTDQPFL

SEQ ID NO: 15 - protein, 137 aa, synthetic construct
  REGION 1..137: note = hTrx.v2-M30
MVKQIESKTAFQEALDAAGDKLVVVDFSATWCGPCKMIKPFFHSLSEKYSNVIFLEVDVDDCQDVASECEVKSMPTFQFFKKGQKVGEFSGANKEKLEATINELVGGGGSPSKPSFQEFVDWENVSPELNSTDQPFL

SEQ ID NO: 16 - protein, 136 aa, synthetic construct
  REGION 1..136: note = hTrx.v1-M30
VKQIESKTAFQEALDAAGDKLVVVDFSATWCGPCKMIKPFFHSLSEKYSNVIFLEVDVDDSQDVASESEVKSMPTFQFFKKGQKVGEFSGANKEKLEATINELVGGGGSPSKPSFQEFVDWENVSPELNSTDQPFL

SEQ ID NO: 17 - protein, 137 aa, synthetic construct
  REGION 1..137: note = hTrx.v1-M30
MVKQIESKTAFQEALDAAGDKLVVVDFSATWCGPCKMIKPFFHSLSEKYSNVIFLEVDVDDSQDVASESEVKSMPTFQFFKKGQKVGEFSGANKEKLEATINELVGGGGSPSKPSFQEFVDWENVSPELNSTDQPFL

SEQ ID NO: 18 - protein, 137 aa, synthetic construct
  REGION 1..137: note = hTrx.v3-M30
MVKQIESKTAFQEALDAAGDKLVVVDFSATWSGPSKMIKPFFHSLSEKYSNVIFLEVDVDDSQDVASESEVKSMPTFQFFKKGQKVGEFSGANKEKLEATINELVGGGGSPSKPSFQEFVDWENVSPELNSTDQPFL

SEQ ID NO: 19 - protein, 141 aa, synthetic construct
  REGION 1..141: note = TrxA.v2-M30
MSDKIIHLTDDSFDTDVLKADGAILVDFWAEWSGPSKMIAPILDEIADEYQGKLTVAKLNIDQNPGTAPKYGIRGIPTLLLFKNGEVAATKVGALSKGQLKEFLDANLAGGGGSPSKPSFQEFVDWENVSPELNSTDQPFL

SEQ ID NO: 20 - protein, 182 aa, synthetic construct
  REGION 1..182: note = hTrx.v3-M30-PSBD
MVKQIESKTAFQEALDAAGDKLVVVDFSATWSGPSKMIKPFFHSLSEKYSNVIFLEVDVDDSQDVASESEVKSMPTFQFFKKGQKVGEFSGANKEKLEATINELVGGGGGPSKPSFQEFVDWENVSPELNSTDQPFLGGGGGVIAMPSVRKYAREKGVDIRLVQGTGKNGRVLKEDIDAWLA

SEQ ID NO: 21 - protein, 137 aa, synthetic construct
  REGION 1..137: note = hTrx.v1-M44
MVKQIESKTAFQEALDAAGDKLVVVDFSATWCGPCKMIKPFFHSLSEKYSNVIFLEVDVDDSQDVASESEVKSMPTFQFFKKGQKVGEFSGANKEKLEATINELVGGGGSEFKHIKAFDRTFANNPGPMVVFATPGM

SEQ ID NO: 22 - protein, 137 aa, synthetic construct
  REGION 1..137: note = hTrx.v2-M44
MVKQIESKTAFQEALDAAGDKLVVVDFSATWCGPCKMIKPFFHSLSEKYSNVIFLEVDVDDCQDVASECEVKSMPTFQFFKKGQKVGEFSGANKEKLEATINELVGGGGSEFKHIKAFDRTFANNPGPMVVFATPGM

SEQ ID NO: 23 - protein, 182 aa, synthetic construct
  REGION 1..182: note = hTrx.v3-M44-PSBD
MVKQIESKTAFQEALDAAGDKLVVVDFSATWSGPSKMIKPFFHSLSEKYSNVIFLEVDVDDSQDVASESEVKSMPTFQFFKKGQKVGEFSGANKEKLEATINELVGGGGGEFKHIKAFDRTFANNPGPMVVFATPGMGGGGGVIAMPSVRKYAREKGVDIRLVQGTGKNGRVLKEDIDAWLA

SEQ ID NO: 24 - protein, 137 aa, synthetic construct
  REGION 1..137: note = hTrx.v3-M12
MVKQIESKTAFQEALDAAGDKLVVVDFSATWSGPSKMIKPFFHSLSEKYSNVIFLEVDVDDSQDVASESEVKSMPTFQFFKKGQKVGEFSGANKEKLEATINELVGGGGSTPPPEEAMPFEFNGPAQGDHSQPPLQV

SEQ ID NO: 25 - protein, 182 aa, synthetic construct
  REGION 1..182: note = hTrx.v3-M12-PSBD
MVKQIESKTAFQEALDAAGDKLVVVDFSATWSGPSKMIKPFFHSLSEKYSNVIFLEVDVDDSQDVASESEVKSMPTFQFFKKGQKVGEFSGANKEKLEATINELVGGGGGTPPPEEAMPFEFNGPAQGDHSQPPLQVGGGGGVIAMPSVRKYAREKGVDIRLVQGTGKNGRVLKEDIDAWLA

SEQ ID NO: 26 - protein, 137 aa, synthetic construct
  REGION 1..137: note = hTrx.v3-M21
MVKQIESKTAFQEALDAAGDKLVVVDFSATWSGPSKMIKPFFHSLSEKYSNVIFLEVDVDDSQDVASESEVKSMPTFQFFKKGQKVGEFSGANKEKLEATINELVGGGGSSSPDEVALVEGVQSLGFTYLRLKDNYM

SEQ ID NO: 27 - protein, 182 aa, synthetic construct
  REGION 1..182: note = hTrx.v3-M21-PSBD
MVKQIESKTAFQEALDAAGDKLVVVDFSATWSGPSKMIKPFFHSLSEKYSNVIFLEVDVDDSQDVASESEVKSMPTFQFFKKGQKVGEFSGANKEKLEATINELVGGGGGSSPDEVALVEGVQSLGFTYLRLKDNYMGGGGGVIAMPSVRKYAREKGVDIRLVQGTGKNGRVLKEDIDAWLA

SEQ ID NO: 28 - protein, 127 aa, synthetic construct
  REGION 1..127: note = hTrx.v3-CT5
MVKQIESKTAFQEALDAAGDKLVVVDFSATWSGPSKMIKPFFHSLSEKYSNVIFLEVDVDDSQDVASESEVKSMPTFQFFKKGQKVGEFSGANKEKLEATINELVGGGGSIYLESVAIMPQLFMVSK

SEQ ID NO: 29 - protein, 172 aa, synthetic construct
  REGION 1..172: note = hTrx.v3-CT5-PSBD
MVKQIESKTAFQEALDAAGDKLVVVDFSATWSGPSKMIKPFFHSLSEKYSNVIFLEVDVDDSQDVASESEVKSMPTFQFFKKGQKVGEFSGANKEKLEATINELVGGGGGIYLESVAIMPQLFMVSKGGGGGVIAMPSVRKYAREKGVDIRLVQGTGKNGRVLKEDIDAWLA

SEQ ID NO: 30 - protein, 137 aa, synthetic construct
  REGION 1..137: note = hTrx.wt-MelanA
MVKQIESKTAFQEALDAAGDKLVVVDFSATWCGPCKMIKPFFHSLSEKYSNVIFLEVDVDDCQDVASECEVKCMPTFQFFKKGQKVGEFSGANKEKLEATINELVGGGGGYPKKGHGHSYTTAEELAGIGILTVILG

SEQ ID NO: 31 - protein, 137 aa, synthetic construct
  REGION 1..137: note = hTrx.v3-MelanA
MVKQIESKTAFQEALDAAGDKLVVVDFSATWSGPSKMIKPFFHSLSEKYSNVIFLEVDVDDSQDVASESEVKSMPTFQFFKKGQKVGEFSGANKEKLEATINELVGGGGGYPKKGHGHSYTTAEELAGIGILTVILG

SEQ ID NO: 32 - protein, 182 aa, synthetic construct
  REGION 1..182: note = hTrx.v3-MelanA-PSBD
MVKQIESKTAFQEALDAAGDKLVVVDFSATWSGPSKMIKPFFHSLSEKYSNVIFLEVDVDDSQDVASESEVKSMPTFQFFKKGQKVGEFSGANKEKLEATINELVGGGGGYPKKGHGHSYTTAEELAGIGILTVILGGGGGGVIAMPSVRKYAREKGVDIRLVQGTGKNGRVLKEDIDAWLA

SEQ ID NO: 33 - protein, 151 aa, synthetic construct
  REGION 1..151: note = pc0735 (TrxA-M30-His)
MSDKIIHLTDDSFDTDVLKADGAILVDFWAEWCGPCKMIAPILDEIADEYQGKLTVAKLNIDQNPGTAPKYGIRGIPTLLLFKNGEVAATKVGALSKGQLKEFLDANLAGGGGSPSKPSFQEFVDWENVSPELNSTDQPFLSSGGHHHHHH

SEQ ID NO: 34 - protein, 145 aa, synthetic construct
  REGION 1..145: note = pc0763 (hTrx.v2-M30-His)
MVKQIESKTAFQEALDAAGDKLVVVDFSATWCGPCKMIKPFFHSLSEKYSNVIFLEVDVDDCQDVASECEVKSMPTFQFFKKGQKVGEFSGANKEKLEATINELVGGGGSPSKPSFQEFVDWENVSPELNSTDQPFLGGHHHHHH

SEQ ID NO: 35 - protein, 145 aa, synthetic construct
  REGION 1..145: note = pc0764 (hTrx.v1-M30-His)
MVKQIESKTAFQEALDAAGDKLVVVDFSATWCGPCKMIKPFFHSLSEKYSNVIFLEVDVDDSQDVASESEVKSMPTFQFFKKGQKVGEFSGANKEKLEATINELVGGGGSPSKPSFQEFVDWENVSPELNSTDQPFLGGHHHHHH

SEQ ID NO: 36 - protein, 145 aa, synthetic construct
  REGION 1..145: note = pc0792 (hTrx.v3-M30-His)
MVKQIESKTAFQEALDAAGDKLVVVDFSATWSGPSKMIKPFFHSLSEKYSNVIFLEVDVDDSQDVASESEVKSMPTFQFFKKGQKVGEFSGANKEKLEATINELVGGGGSPSKPSFQEFVDWENVSPELNSTDQPFLGGHHHHHH

SEQ ID NO: 37 - protein, 149 aa, synthetic construct
  REGION 1..149: note = pc0802 (TrxA.v2-M30-His)
MSDKIIHLTDDSFDTDVLKADGAILVDFWAEWSGPSKMIAPILDEIADEYQGKLTVAKLNIDQNPGTAPKYGIRGIPTLLLFKNGEVAATKVGALSKGQLKEFLDANLAGGGGSPSKPSFQEFVDWENVSPELNSTDQPFLGGHHHHHH

SEQ ID NO: 38 - protein, 190 aa, synthetic construct
  REGION 1..190: note = pc0890 (hTrx.v3-M30-PSBD-His)
MVKQIESKTAFQEALDAAGDKLVVVDFSATWSGPSKMIKPFFHSLSEKYSNVIFLEVDVDDSQDVASESEVKSMPTFQFFKKGQKVGEFSGANKEKLEATINELVGGGGGPSKPSFQEFVDWENVSPELNSTDQPFLGGGGGVIAMPSVRKYAREKGVDIRLVQGTGKNGRVLKEDIDAWLAGGHHHHHH

SEQ ID NO: 39 - protein, 147 aa, synthetic construct
  REGION 1..147: note = pc0761 (hTrx.v1-M44-His)
MVKQIESKTAFQEALDAAGDKLVVVDFSATWCGPCKMIKPFFHSLSEKYSNVIFLEVDVDDSQDVASESEVKSMPTFQFFKKGQKVGEFSGANKEKLEATINELVGGGGSEFKHIKAFDRTFANNPGPMVVFATPGMSSGGHHHHHH

SEQ ID NO: 40 - protein, 147 aa, synthetic construct
  REGION 1..147: note = pc0762 (hTrx.v2-M44-His)
MVKQIESKTAFQEALDAAGDKLVVVDFSATWCGPCKMIKPFFHSLSEKYSNVIFLEVDVDDCQDVASECEVKSMPTFQFFKKGQKVGEFSGANKEKLEATINELVGGGGSEFKHIKAFDRTFANNPGPMVVFATPGMSSGGHHHHHH

SEQ ID NO: 41 - protein, 190 aa, synthetic construct
  REGION 1..190: note = pc0895 (hTrx.v3-M44-PSBD-His)
MVKQIESKTAFQEALDAAGDKLVVVDFSATWSGPSKMIKPFFHSLSEKYSNVIFLEVDVDDSQDVASESEVKSMPTFQFFKKGQKVGEFSGANKEKLEATINELVGGGGGEFKHIKAFDRTFANNPGPMVVFATPGMGGGGGVIAMPSVRKYAREKGVDIRLVQGTGKNGRVLKEDIDAWLAGGHHHHHH

SEQ ID NO: 42 - protein, 145 aa, synthetic construct
  REGION 1..145: note = pc0811 (hTrx.v3-M12-His)
MVKQIESKTAFQEALDAAGDKLVVVDFSATWSGPSKMIKPFFHSLSEKYSNVIFLEVDVDDSQDVASESEVKSMPTFQFFKKGQKVGEFSGANKEKLEATINELVGGGGSTPPPEEAMPFEFNGPAQGDHSQPPLQVGGHHHHHH

SEQ ID NO: 43 - protein, 190 aa, synthetic construct
  REGION 1..190: note = pc0883 (hTrx.v3-M12-PSBD-His)
MVKQIESKTAFQEALDAAGDKLVVVDFSATWSGPSKMIKPFFHSLSEKYSNVIFLEVDVDDSQDVASESEVKSMPTFQFFKKGQKVGEFSGANKEKLEATINELVGGGGGTPPPEEAMPFEFNGPAQGDHSQPPLQVGGGGGVIAMPSVRKYAREKGVDIRLVQGTGKNGRVLKEDIDAWLAGGHHHHHH

SEQ ID NO: 44 - protein, 145 aa, synthetic construct
  REGION 1..145: note = pc0812 (hTrx.v3-M21-His)
MVKQIESKTAFQEALDAAGDKLVVVDFSATWSGPSKMIKPFFHSLSEKYSNVIFLEVDVDDSQDVASESEVKSMPTFQFFKKGQKVGEFSGANKEKLEATINELVGGGGSSSPDEVALVEGVQSLGFTYLRLKDNYMGGHHHHHH

SEQ ID NO: 45 - protein, 190 aa, synthetic construct
  REGION 1..190: note = pc0869 (hTrx.v3-M21-PSBD-His)
MVKQIESKTAFQEALDAAGDKLVVVDFSATWSGPSKMIKPFFHSLSEKYSNVIFLEVDVDDSQDVASESEVKSMPTFQFFKKGQKVGEFSGANKEKLEATINELVGGGGGSSPDEVALVEGVQSLGFTYLRLKDNYMGGGGGVIAMPSVRKYAREKGVDIRLVQGTGKNGRVLKEDIDAWLAGGHHHHHH

SEQ ID NO: 46 - protein, 135 aa, synthetic construct
  REGION 1..135: note = pc0824 (hTrx.v3-CT5-His)
MVKQIESKTAFQEALDAAGDKLVVVDFSATWSGPSKMIKPFFHSLSEKYSNVIFLEVDVDDSQDVASESEVKSMPTFQFFKKGQKVGEFSGANKEKLEATINELVGGGGSIYLESVAIMPQLFMVSKGGHHHHHH

SEQ ID NO: 47 - protein, 180 aa, synthetic construct
  REGION 1..180: note = pc0886 (hTrx.v3-CT5-PSBD-His)
MVKQIESKTAFQEALDAAGDKLVVVDFSATWSGPSKMIKPFFHSLSEKYSNVIFLEVDVDDSQDVASESEVKSMPTFQFFKKGQKVGEFSGANKEKLEATINELVGGGGGIYLESVAIMPQLFMVSKGGGGGVIAMPSVRKYAREKGVDIRLVQGTGKNGRVLKEDIDAWLAGGHHHHHH

SEQ ID NO: 48 - protein, 145 aa, synthetic construct
  REGION 1..145: note = pc0993 (hTrx.wt-MelanA-His)
MVKQIESKTAFQEALDAAGDKLVVVDFSATWCGPCKMIKPFFHSLSEKYSNVIFLEVDVDDCQDVASECEVKCMPTFQFFKKGQKVGEFSGANKEKLEATINELVGGGGGYPKKGHGHSYTTAEELAGIGILTVILGGGHHHHHH

SEQ ID NO: 49 - protein, 145 aa, synthetic construct
  REGION 1..145: note = pc0992 (hTrx.v3-MelanA-His)
MVKQIESKTAFQEALDAAGDKLVVVDFSATWSGPSKMIKPFFHSLSEKYSNVIFLEVDVDDSQDVASESEVKSMPTFQFFKKGQKVGEFSGANKEKLEATINELVGGGGGYPKKGHGHSYTTAEELAGIGILTVILGGGHHHHHH

SEQ ID NO: 50 - protein, 190 aa, synthetic construct
  REGION 1..190: note = pc0984 (hTrx.v3-MelanA-PSBD-His)
MVKQIESKTAFQEALDAAGDKLVVVDFSATWSGPSKMIKPFFHSLSEKYSNVIFLEVDVDDSQDVASESEVKSMPTFQFFKKGQKVGEFSGANKEKLEATINELVGGGGGYPKKGHGHSYTTAEELAGIGILTVILGGGGGGVIAMPSVRKYAREKGVDIRLVQGTGKNGRVLKEDIDAWLAGGHHHHHH

SEQ ID NO: 51 - protein, 5 aa, synthetic construct
  REGION 1..5: note = GS linker 1
GGGGS

SEQ ID NO: 52 - protein, 4 aa, synthetic construct
  REGION 1..4: note = GS linker 2
SSGG

SEQ ID NO: 53 - skipped

SEQ ID NO: 54 - protein, 5 aa, synthetic construct
  REGION 1..5: note = GS linker 4
GGGGG

SEQ ID NO: 55 - DNA, 255 bp, synthetic construct
  misc_feature 1..255: note = hTrx.v1 backbone nucleotide sequence
  source 1..255: mol_type = other DNA
atggttaaacaaattgagtcgaaaaccgccttccaagaagctcttgatgctgctggtgataagttggtcgtagttgacttctcagccacttggtgcggtccatgcaaaatgataaagccttttttccactcgttgagtgagaagtattcaaacgtaatttttttagaagtggatgtcgatgattcacaagatgttgcaagtgagagcgaagtcaagtctatgcccacgtttcaatttttcaaaaaaggtcagaag

SEQ ID NO: 56 - DNA, 255 bp, synthetic construct
  misc_feature 1..255: note = hTrx.v2 backbone nucleotide sequence
  source 1..255: mol_type = other DNA
atggttaaacaaattgagtcgaaaaccgccttccaagaagctcttgatgctgctggtgataagttggtcgtagttgacttctcagccacttggtgcggtccatgcaaaatgataaagccttttttccactcgttgagtgagaagtattcaaacgtaatttttttagaagtggatgtcgatgattgccaagatgttgcaagtgagtgcgaagtcaagtctatgcccacgtttcaatttttcaaaaaaggtcagaag

SEQ ID NO: 57 - DNA, 255 bp, synthetic construct
  misc_feature 1..255: note = hTrx.v3 backbone nucleotide sequence
  source 1..255: mol_type = other DNA
atggttaaacaaattgagtcgaaaaccgccttccaagaagctcttgatgctgctggtgataagttggtcgtagttgacttctcagccacttggtctggtccatctaaaatgataaagccttttttccactcgttgagtgagaagtattcaaacgtaatttttttagaagtggatgtcgatgattcacaagatgttgcaagtgagagcgaagtcaagtctatgcccacgtttcaatttttcaaaaaaggtcagaag

SEQ ID NO: 58 - DNA, 255 bp, synthetic construct
  misc_feature 1..255: note = TrxA backbone nucleotide sequence
  source 1..255: mol_type = other DNA
atgagcgataaaattattcacctgactgacgacagttttgacacggatgtactcaaagcggacggggcgatcctcgtcgatttctgggcagagtggtgcggtccgtgcaaaatgatcgccccgattctggatgaaatcgctgacgaatatcagggcaaactgaccgttgcaaaactgaacatcgatcaaaaccctggcactgcgccgaaatatggcatccgtggtatcccgactctgctgctgttcaaaaacggt

SEQ ID NO: 59 - DNA, 255 bp, synthetic construct
  misc_feature 1..255: note = TrxA.v2 backbone nucleotide sequence
  source 1..255: mol_type = other DNA
atgagcgataaaattattcacctgactgacgacagttttgacacggatgtactcaaagcggacggggcgatcctcgtcgatttctgggcagagtggtctggtccgtctaaaatgatcgccccgattctggatgaaatcgctgacgaatatcagggcaaactgaccgttgcaaaactgaacatcgatcaaaaccctggcactgcgccgaaatatggcatccgtggtatcccgactctgctgctgttcaaaaacggt

SEQ ID NO: 60 - DNA, 120 bp, synthetic construct
  misc_feature 1..120: note = PSBD backbone nucleotide sequence
  source 1..120: mol_type = other DNA
gttatcgctatgccgtccgtacgcaaatatgcacgtgaaaaaggcgttgatatccgcctggttcagggtaccggtaaaaacggccgtgttctgaaagaagacatcgacgcgtggctggct

SEQ ID NO: 61 - DNA, 65 bp, synthetic construct
  misc_feature 1..65: note = backbone Forward1 primer
  source 1..65: mol_type = other DNA
gcgtctagaaataattttgtttaactttaagaaggagatatacatatggcagatctcaattggat

SEQ ID NO: 62 - DNA, 25 bp, synthetic construct
  misc_feature 1..25: note = backbone Reverse1 primer
  source 1..25: mol_type = other DNA
cagcggtttctttaccagactcgag

SEQ ID NO: 63 - DNA, 58 bp, synthetic construct
  misc_feature 1..58: note = TrxA Forward SpeI primer
  source 1..58: mol_type = other DNA
gcgactagtaataattttgtttaactttaagaaggagatatacatatgagcgataaaa

SEQ ID NO: 64 - DNA, 39 bp, synthetic construct
  misc_feature 1..39: note = TrxA Forward SS mut
  source 1..39: mol_type = other DNA
tggtctggtccgtctaaaatgatcgccccgattctggat

SEQ ID NO: 65 - DNA, 40 bp, synthetic construct
  misc_feature 1..40: note = TrxA Reverse SS mut
  source 1..40: mol_type = other DNA
cattttagacggaccagaccactctgcccagaaatcgacg

SEQ ID NO: 66 - DNA, 33 bp, synthetic construct
  misc_feature 1..33: note = TrxA BamHI Reverse primer
  source 1..33: mol_type = other DNA
gcgggatccaccaccaccggccaggttagcgtc

SEQ ID NO: 67 - DNA, 85 bp, synthetic construct
  misc_feature 1..85: note = M30 Forward primer
  source 1..85: mol_type = other DNA
aggaccgagcaaaccgtcgtttcaggaatttgtggactgggaaaacgtgtcgccggaactgaacagcaccgatcagccgtttctg

SEQ ID NO: 68 - DNA, 85 bp, synthetic construct
  misc_feature 1..85: note = M30 Reverse primer
  source 1..85: mol_type = other DNA
cacccagaaacggctgatcggtgctgttcagttccggcgacacgttttcccagtccacaaattcctgaaacgacggtttgctcgg

SEQ ID NO: 69 - DNA, 88 bp, synthetic construct
  misc_feature 1..88: note = PSBD Forward primer
  source 1..88: mol_type = other DNA
gcaaatatgcacgtgaaaaaggcgttgatatccgcctggttcagggtaccggtaaaaacggccgtgttctgaaagaagacatcgacgc

SEQ ID NO: 70 - DNA, 74 bp, synthetic construct
  misc_feature 1..74: note = PSBD Reverse primer
  source 1..74: mol_type = other DNA
cgacgagctctcaatggtggtgatggtgatgtccgccagccagccacgcgtcgatgtcttctttcagaacacgg

SEQ ID NO: 71 - DNA, 32 bp, synthetic construct
  misc_feature 1..32: note = hT NdeI Forward primer
  source 1..32: mol_type = other DNA
gcgcatatggttaaacaaattgagtcgaaaac

SEQ ID NO: 72 - DNA, 48 bp, synthetic construct
  misc_feature 1..48: note = hTrx.v3 Reverse primer
  source 1..48: mol_type = other DNA
tatcattttagatggaccagaccaagtggctgagaagtcaactacgac

SEQ ID NO: 73 - DNA, 51 bp, synthetic construct
  misc_feature 1..51: note = hTrx.v3 Forward primer
  source 1..51: mol_type = other DNA
cacttggtctggtccatctaaaatgataaagccttttttccactcgttgag

SEQ ID NO: 74 - DNA, 47 bp, synthetic construct
  misc_feature 1..47: note = hT BsaI Reverse1 primer
  source 1..47: mol_type = other DNA
tgagacccagcgttgcgggtctcttcctccaccaccaccgaccagtt

SEQ ID NO: 75 - DNA, 89 bp, synthetic construct
  misc_feature 1..89: note = hT BsaI Reverse2 primer
  source 1..89: mol_type = other DNA
ccggtaccctgaaccaggcggatatcaacgcctttttcacgtgcatatttgcgtacggacggcatagcgataactcctccaccaccacc

SEQ ID NO: 76 - DNA, 48 bp, synthetic construct
  misc_feature 1..48: note = BsaI Forward primer
  source 1..48: mol_type = other DNA
agagacccgcaacgctgggtctcaggtggtggtggaggagttatcgct

SEQ ID NO: 77 - DNA, 85 bp, synthetic construct
  misc_feature 1..85: note = M44 Forward primer
  source 1..85: mol_type = other DNA
aggagaatttaaacatattaaagcgtttgatcgtacctttgcgaataacccgggtccgatggtggtgtttgcgaccccgggtatg

SEQ ID NO: 78 - DNA, 85 bp, synthetic construct
  misc_feature 1..85: note = M44 Reverse primer
  source 1..85: mol_type = other DNA
cacccatacccggggtcgcaaacaccaccatcggacccgggttattcgcaaaggtacgatcaaacgctttaatatgtttaaattc

SEQ ID NO: 79 - DNA, 85 bp, synthetic construct
  misc_feature 1..85: note = M12 Forward primer
  source 1..85: mol_type = other DNA
aggaaccccgccgccggaagaagcgatgccgtttgaatttaatggtccggcgcagggtgatcatagccagccgccgctgcaggtg

SEQ ID NO: 80 - DNA, 85 bp, synthetic construct
  misc_feature 1..85: note = M12 Reverse primer
  source 1..85: mol_type = other DNA
cacccacctgcagcggcggctggctatgatcaccctgcgccggaccattaaattcaaacggcatcgcttcttccggcggcggggt

SEQ ID NO: 81 - DNA, 85 bp, synthetic construct
  misc_feature 1..85: note = M21 Forward primer
  source 1..85: mol_type = other DNA
aggaagcagcccggatgaagtggcgctggttgaaggtgtgcagagcctgggttttacctatctgcgtctgaaagataattatatg

SEQ ID NO: 82 - DNA, 85 bp, synthetic construct
  misc_feature 1..85: note = M21 Reverse primer
  source 1..85: mol_type = other DNA
cacccatataattatctttcagacgcagataggtaaaacccaggctctgcacaccttcaaccagcgccacttcatccgggctgct

SEQ ID NO: 83 - DNA, 55 bp, synthetic construct
  misc_feature 1..55: note = CT5 Forward primer
  source 1..55: mol_type = other DNA
aggaatttatctggaaagcgtggcgattatgccgcagctgtttatggtgagcaaa

SEQ ID NO: 84 - DNA, 55 bp, synthetic construct
  misc_feature 1..55: note = CT5 Reverse primer
  source 1..55: mol_type = other DNA
cacctttgctcaccataaacagctgcggcataatcgccacgctttccagataaat

SEQ ID NO: 85 - DNA, 85 bp, synthetic construct
  misc_feature 1..85: note = MelanA Forward primer
  source 1..85: mol_type = other DNA
aggatatccgaaaaaaggccatggccatagctataccaccgcggaagaactggcgggcattggcattctgaccgtgattctgggc

SEQ ID NO: 86 - DNA, 85 bp, synthetic construct
  misc_feature 1..85: note = MelanA Reverse primer
  source 1..85: mol_type = other DNA
caccgcccagaatcacggtcagaatgccaatgcccgccagttcttccgcggtggtatagctatggccatggccttttttcggata

SEQ ID NO: 87 - DNA, 25 bp, synthetic construct
  misc_feature 1..25: note = T7 Forward primer
  source 1..25: mol_type = other DNA
gtccggcgtagaggatcgagatctc

SEQ ID NO: 88 - DNA, 63 bp, synthetic construct
  misc_feature 1..63: note = MelanA wt Reverse primer
  source 1..63: mol_type = other DNA
gcggagctctcaatggtggtgatggtgatgtccgccttctttcgcaattttgtttttcgcgcg

SEQ ID NO: 89 - DNA, 48 bp, synthetic construct
  misc_feature 1..48: note = hTrx wt Forward primer
  source 1..48: mol_type = other DNA
tgcgaagtcaagtgcatgcccacgtttcaatttttcaaaaaaggtcag

SEQ ID NO: 90 - DNA, 44 bp, synthetic construct
  misc_feature 1..44: note = hTrx wt Reverse primer
  source 1..44: mol_type = other DNA
tgaaacgtgggcatgcacttgacttcgcactcacttgcaacatc